European Patent Specification EP 3 765 507 B1, published April 24, 2024. Title: ANTI-CD25 ANTIBODY AGENTS. Applicant: TUSK THERAPEUTICS LTD CANCER RESEARCH TECHNOLOGY LIMITED. The sequence listing filed with the application follows.

SEQUENCE LISTING (17 sequences)

SEQ ID NO: 1 - protein, 10 aa, homo sapiens
GFTLDSYGVS

SEQ ID NO: 2 - protein, 14 aa, homo sapiens
VTSSGGSAYYADSV

SEQ ID NO: 3 - protein, 17 aa, homo sapiens
DRYVYTGGYLYHYGMDL

SEQ ID NO: 4 - protein, 11 aa, homo sapiens
RASQSISDYLA

SEQ ID NO: 5 - protein, 8 aa, homo sapiens
YAASTLPF

SEQ ID NO: 6 - protein, 12 aa, homo sapiens
QGTYDSSDWYWA

SEQ ID NO: 7 - protein, 125 aa, homo sapiens
EVQLVESGGGLIQPGGSLRLSCAASGFTLDSYGVSWVRQAPGKGLEWVGVTSSGGSAYYADSVKGRFTISRDNSKNTLYLQMNSLRAEDTAVYYCARDRYVYTGGYLYHYGMDLWGQGTLVTVSS

SEQ ID NO: 8 - protein, 110 aa, homo sapiens
DIQMTQSPSSLSASVGDRVTITCRASQSISDYLAWYQQKPGKVPKLLIYAASTLPFGVPSRFSGSGSGTDFTLTISSLQPEDVATYYCQGTYDSSDWYWAFGGGTKVEIK

SEQ ID NO: 9 - protein, 10 aa, homo sapiens
GFSVDIYDMS

SEQ ID NO: 10 - protein, 15 aa, homo sapiens
YISSSLGATYYADSV

SEQ ID NO: 11 - protein, 16 aa, homo sapiens
ERIYSVYTLDYYAMDL

SEQ ID NO: 12 - protein, 11 aa, homo sapiens
QASQGITNNLN

SEQ ID NO: 13 - protein, 8 aa, homo sapiens
YAASTLQS

SEQ ID NO: 14 - protein, 12 aa, homo sapiens
QQGYTTSNVDNA

SEQ ID NO: 15 - protein, 125 aa, homo sapiens
EVQLLESGGGLVQPGGSLRLSCAASGFSVDIYDMSWVRQAPGKGLEWVAYISSSLGATYYADSVKGRFTISRDNSKNTLYLQMNSLRAEDTAVYYCARERIYSVYTLDYYAMDLWGQGTLVTVSS

SEQ ID NO: 16 - protein, 110 aa, homo sapiens
DIQMTQSPSSLSASVGDRVTITCQASQGITNNLNWYQQKPGKVPKLLIYAASTLQSGVPSRFSGSGSGTDFTLTISSLQPEDVATYYCQQGYTTSNVDNAFGGGTKVEIK

SEQ ID NO: 17 - protein, 272 aa, homo sapiens
MDSYLLMWGLLTFIMVPGCQAELCDDDPPEIPHATFKAMAYKEGTMLNCECKRGFRRIKSGSLYMLCTGNSSHSSWDNQCQCTSSATRNTTKQVTPQPEEQKERKTTEMQSPMQPVDQASLPGHCREPPPWENEATERIYHFVVGQMVYYQCVQGYRALHRGPAESVCKMTHGKTRWTQPQLICTGEMETSQFPGEEKPQASPEGRPESETSCLVTTTDFQIQTEMAATMETSIFTTEYQVAVAGCVFLLISVLLLSGLTWQRRQRKSRRTI